European Patent Specification EP 4 012 019 B1, published February 21, 2024. Title: Bifidobacterium breve 207-1 and use thereof. Applicant: ByHealth Co.,Ltd. The sequence listing filed with the application follows.

SEQUENCE LISTING (19 sequences)

SEQ ID NO: 1 - DNA, 17 bp, artificial
  primer
ctcctggaaacgggtgg

SEQ ID NO: 2 - DNA, 22 bp, artificial
  primer
ggtgttcttcccgatatctaca

SEQ ID NO: 3 - DNA, 19 bp, artificial
  primer
ctccagttggatgcatgtc

SEQ ID NO: 4 - DNA, 18 bp, artificial
  primer
tccagttgaccgcatggt

SEQ ID NO: 5 - DNA, 18 bp, artificial
  primer
cgaaggcttgctcccagt

SEQ ID NO: 6 - DNA, 19 bp, artificial
  primer
cagtccatcgcatggtggt

SEQ ID NO: 7 - DNA, 18 bp, artificial
  primer
gaaggcttgctccccaac

SEQ ID NO: 8 - DNA, 21 bp, artificial
  primer
ccacatgatcgcatgtgattg

SEQ ID NO: 9 - DNA, 19 bp, artificial
  primer
ccgaaggcttgctcccaaa

SEQ ID NO: 10 - DNA, 18 bp, artificial
  primer
ccggatgctccatcacac

SEQ ID NO: 11 - DNA, 19 bp, artificial
  primer
acaaagtgccttgctccct

SEQ ID NO: 12 - DNA, 17 bp, artificial
  primer
cggatgctccgactcct

SEQ ID NO: 13 - DNA, 18 bp, artificial
  primer
cgaaggcttgctcccgat

SEQ ID NO: 14 - DNA, 20 bp, artificial
  primer
ttccagttgatcgcatggtc

SEQ ID NO: 15 - DNA, 20 bp, artificial
  primer
gggaagccgtatctctacga

SEQ ID NO: 16 - DNA, 20 bp, artificial
  primer
ttccagttgatcgcatggtc

SEQ ID NO: 17 - DNA, 20 bp, artificial
  primer
ggaaaccccatctctgggat

SEQ ID NO: 18 - DNA, 17 bp, artificial
  primer
atcccgggggttcgcct

SEQ ID NO: 19 - DNA, 17 bp, artificial
  primer
gaagggcttgctcccga